European Patent Application EP 4 112 746 A1, published January 4, 2023. Title: Method for predicting a clinical response towards an immune checkpoint inhibitor based on pretreatment therewith. Applicant: Stratifyer Molecular Pathology GmbH. The sequence listing filed with the application follows.

SEQUENCE LISTING (42 sequences)

SEQ ID NO: 1 - DNA, 23 bp, Artificial Sequence
  primer or probe sequence
acccctcagccgtgcctgtgttc

SEQ ID NO: 2 - DNA, 17 bp, Artificial Sequence
  primer or probe sequence
ggccagcccctgaagga

SEQ ID NO: 3 - DNA, 22 bp, Artificial Sequence
  primer or probe sequence
ggaaatccagctccccatagtc

SEQ ID NO: 4 - DNA, 22 bp, Artificial Sequence
  primer or probe sequence
tgagccccagcaaccagacgga

SEQ ID NO: 5 - DNA, 21 bp, Artificial Sequence
  primer or probe sequence
caacacatcggagagcttcgt

SEQ ID NO: 6 - DNA, 16 bp, Artificial Sequence
  primer or probe sequence
ggaaggcggccagctt

SEQ ID NO: 7 - DNA, 26 bp, Artificial Sequence
  primer or probe sequence
cagaagtgccctttgcctccactcaa

SEQ ID NO: 8 - DNA, 23 bp, Artificial Sequence
  primer or probe sequence
ccctaatttgagggtcagttcct

SEQ ID NO: 9 - DNA, 25 bp, Artificial Sequence
  primer or probe sequence
ctcagtcatgcagaaaacaaattga

SEQ ID NO: 10 - DNA, 30 bp, Artificial Sequence
  primer or probe sequence
caaagtgatacacatttggaggagacgtaa

SEQ ID NO: 11 - DNA, 23 bp, Artificial Sequence
  primer or probe sequence
tggcatccaagatacaaactcaa

SEQ ID NO: 12 - DNA, 24 bp, Artificial Sequence
  primer or probe sequence
ttgaagatcagaagttccaatgct

SEQ ID NO: 13 - DNA, 27 bp, Artificial Sequence
  primer or probe sequence
caaagctctgtgcctctgtaatcggca

SEQ ID NO: 14 - DNA, 15 bp, Artificial Sequence
  primer or probe sequence
caccgcggccatcct

SEQ ID NO: 15 - DNA, 19 bp, Artificial Sequence
  primer or probe sequence
agtttgggatccagcaggc

SEQ ID NO: 16 - DNA, 30 bp, Artificial Sequence
  primer or probe sequence
acatcaaggttctgcccacatggtccaccc

SEQ ID NO: 17 - DNA, 21 bp, Artificial Sequence
  primer or probe sequence
gtggcagtgtctgctgagtga

SEQ ID NO: 18 - DNA, 19 bp, Artificial Sequence
  primer or probe sequence
agcacaatcagggccattg

SEQ ID NO: 19 - DNA, 20 bp, Artificial Sequence
  primer or probe sequence
ttcctgccagcgaagcccac

SEQ ID NO: 20 - DNA, 25 bp, Artificial Sequence
  primer or probe sequence
tgagcaactccatcatgtacttcag

SEQ ID NO: 21 - DNA, 15 bp, Artificial Sequence
  primer or probe sequence
ggcgccggtgttggt

SEQ ID NO: 22 - DNA, 21 bp, Artificial Sequence
  primer or probe sequence
caaatgtcccccggcctgtgg

SEQ ID NO: 23 - DNA, 21 bp, Artificial Sequence
  primer or probe sequence
cacaggaaccgaagacgtgtt

SEQ ID NO: 24 - DNA, 19 bp, Artificial Sequence
  primer or probe sequence
gggcttgtctcccgatttg

SEQ ID NO: 25 - DNA, 25 bp, Artificial Sequence
  primer or probe sequence
tccacctcgacctgctctccctgag

SEQ ID NO: 26 - DNA, 22 bp, Artificial Sequence
  primer or probe sequence
cagcaactcgagcatcattctt

SEQ ID NO: 27 - DNA, 21 bp, Artificial Sequence
  primer or probe sequence
gcaggagaaactttgcccaaa

SEQ ID NO: 28 - DNA, 31 bp, Artificial Sequence
  primer or probe sequence
tgctcaaagggagcagatctgagcctgagac

SEQ ID NO: 29 - DNA, 20 bp, Artificial Sequence
  primer or probe sequence
tgctgaggatgctggagtga

SEQ ID NO: 30 - DNA, 25 bp, Artificial Sequence
  primer or probe sequence
gaacattcagtgactccatctacca

SEQ ID NO: 31 - DNA, 22 bp, Artificial Sequence
  primer or probe sequence
tcgcgtctcggaaaccggtagc

SEQ ID NO: 32 - DNA, 20 bp, Artificial Sequence
  primer or probe sequence
gagcgagctgagtggttgtg

SEQ ID NO: 33 - DNA, 21 bp, Artificial Sequence
  primer or probe sequence
agtcagttggtcagccatgct

SEQ ID NO: 34 - DNA, 28 bp, Artificial Sequence
  primer or probe sequence
atgatgctgcttacatgtctcgatccca

SEQ ID NO: 35 - DNA, 23 bp, Artificial Sequence
  primer or probe sequence
tgactttgtcacagcccaagata

SEQ ID NO: 36 - DNA, 20 bp, Artificial Sequence
  primer or probe sequence
aatgcggcatcttcaaacct

SEQ ID NO: 37 - DNA, 28 bp, Artificial Sequence
  primer or probe sequence
ctggacgtacaataccacttccgctgtc

SEQ ID NO: 38 - DNA, 21 bp, Artificial Sequence
  primer or probe sequence
tgtggttcctgcatgaagaca

SEQ ID NO: 39 - DNA, 21 bp, Artificial Sequence
  primer or probe sequence
cagtcttctgatggcggactt

SEQ ID NO: 40 - DNA, 23 bp, Artificial Sequence
  primer or probe sequence
ccctgtcttctgcaaagcaatgc

SEQ ID NO: 41 - DNA, 19 bp, Artificial Sequence
  Primer or Probe Sequence
ggccctgcactctcctgtt

SEQ ID NO: 42 - DNA, 20 bp, Artificial Sequence
  Primer or Probe sequence
agtggctttgcctggagatg